European Patent Specification EP 3 405 790 B1, published June 28, 2023. Title: Transgenic mouse expressing human cereblon. Applicant: Celgene Corporation. Application TBA. The sequence listing filed with the application follows.

SEQUENCE LISTING (17 sequences)

SEQ ID NO: 1 - protein, 442 aa, Homo sapiens [sequence omitted]

SEQ ID NO: 2 - protein, 441 aa, homo sapiens
  amino acid sequence of human CRBN isoform 2
MAGEGDQQDAAHNMGNHLPLLPESEEEDEMEVEDQDSKEAKKPNIINFDTSLPTSHTYLGADMEEFHGRTLHDDDSCQVIPVLPQVMMILIPGQTLPLQLFHPQEVSMVRNLIQKDRTFAVLAYSNVQEREAQFGTTAEIYAYREEQDFGIEIVKVKAIGRQRFKVLELRTQSDGIQQAKVQILPECVLPSTMSAVQLESLNKCQIFPSKPVSREDQCSYKWWQKYQKRKFHCANLTSWPRWLYSLYDAETLMDRIKKQLREWDENLKDDSLPSNPIDFSYRVAACLPIDDVLRIQLLKIGSAIQRLRCELDIMNKCTSLCCKQCQETEITTKNEIFSLSLCGPMAAYVNPHGYVHETLTVYKACNLNLIGRPSTEHSWFPGYAWTVAQCKICASHIGWKFTATKKDMSPQKFWGLTRSALLPTIPDTEDEISPDKVILCL

SEQ ID NO: 3 - protein, 444 aa, mouse
  amino acid sequence of mouse CRBN isoform 1
MAGEGDQQDAAHNMGNHLPLLPDSEDEDDEIEMEVEDQDSKEARKPNIINFDTSLPTSHTYLGADMEEFHGRTLHDDDSCQVIPVLPEVLMILIPGQTLPLQLSHPQEVSMVRNLIQKDRTFAVLAYSNVQEREAQFGTTAEIYAYREEQEFGIEVVKVKAIGRQRFKVLELRTQSDGIQQAKVQILPECVLPSTMSAVQLESLNKCQVFPSKPISWEDQYSCKWWQKYQKRKFHCANLTSWPRWLYSLYDAETLMDRIKKQLREWDENLKDDSLPENPIDFSYRVAACLPIDDVLRIQLLKIGSAIQRLRCELDIMNKCTSLCCKQCQETEITTKNEIFSLSLCGPMAAYVNPHGYVHETLTVYKASNLNLIGRPSTVHSWFPGYAWTIAQCKICASHIGWKFTATKKDMSPQKFWGLTRSALLPTIPETEDEISPDKVILCL

SEQ ID NO: 4 - protein, 445 aa, mouse
  amino acid sequence of mouse CRBN isoform 2
MAGEGDQQDAAHNMGNHLPLLPADSEDEDDEIEMEVEDQDSKEARKPNIINFDTSLPTSHTYLGADMEEFHGRTLHDDDSCQVIPVLPEVLMILIPGQTLPLQLSHPQEVSMVRNLIQKDRTFAVLAYSNVQEREAQFGTTAEIYAYREEQEFGIEVVKVKAIGRQRFKVLELRTQSDGIQQAKVQILPECVLPSTMSAVQLESLNKCQVFPSKPISWEDQYSCKWWQKYQKRKFHCANLTSWPRWLYSLYDAETLMDRIKKQLREWDENLKDDSLPENPIDFSYRVAACLPIDDVLRIQLLKIGSAIQRLRCELDIMNKCTSLCCKQCQETEITTKNEIFSLSLCGPMAAYVNPHGYVHETLTVYKASNLNLIGRPSTVHSWFPGYAWTIAQCKICASHIGWKFTATKKDMSPQKFWGLTRSALLPTIPETEDEISPDKVILCL

SEQ ID NO: 5 - DNA, 1329 bp, Homo sapiens
  cDNA sequence encoding human CRBN isoform 1
atggccggcgaaggagatcagcaggacgctgcgcacaacatgggcaaccacctgccgctcctgcctgcagagagtgaggaagaagatgaaatggaagttgaagaccaggatagtaaagaagccaaaaaaccaaacatcataaattttgacaccagtctgccgacatcacatacatacctaggtgctgatatggaagaatttcatggcaggactttgcacgatgacgacagctgtcaggtgattccagttcttccacaagtgatgatgatcctgattcccggacagacattacctcttcagctttttcaccctcaagaagtcagtatggtgcggaatttaattcagaaagatagaacctttgctgttcttgcatacagcaatgtacaggaaagggaagcacagtttggaacaacagcagagatatatgcctatcgagaagaacaggattttggaattgagatagtgaaagtgaaagcaattggaagacaaaggttcaaagtccttgagctaagaacacagtcagatggaatccagcaagctaaagtgcaaattcttcccgaatgtgtgttgccttcaaccatgtctgcagttcaattagaatccctcaataagtgccagatatttccttcaaaacctgtctcaagagaagaccaatgttcatataaatggtggcagaaataccagaagagaaagtttcattgtgcaaatctaacttcatggcctcgctggctgtattccttatatgatgctgagaccttaatggacagaatcaagaaacagctacgtgaatgggatgaaaatctaaaagatgattctcttccttcaaatccaatagatttttcttacagagtagctgcttgtcttcctattgatgatgtattgagaattcagctccttaaaattggcagtgctatccagcgacttcgctgtgaattagacattatgaataaatgtacttccctttgctgtaaacaatgtcaagaaacagaaataacaaccaaaaatgaaatattcagtttatccttatgtgggccgatggcagcttatgtgaatcctcatggatatgtgcatgagacacttactgtgtataaggcttgcaacttgaatctgataggccggccttctacagaacacagctggtttcctgggtatgcctggactgttgcccagtgtaagatctgtgcaagccatattggatggaagtttacggccaccaaaaaagacatgtcacctcaaaaattttggggcttaacgcgatctgctctgttgcccacgatcccagacactgaagatgaaataagtccagacaaagtaatactttgcttgtaa

SEQ ID NO: 6 - DNA, 1326 bp, Homo sapiens
  cDNA sequence encoding human CRBN isoform 2
atggccggcgaaggagatcagcaggacgctgcgcacaacatgggcaaccacctgccgctcctgcctgagagtgaggaagaagatgaaatggaagttgaagaccaggatagtaaagaagccaaaaaaccaaacatcataaattttgacaccagtctgccgacatcacatacatacctaggtgctgatatggaagaatttcatggcaggactttgcacgatgacgacagctgtcaggtgattccagttcttccacaagtgatgatgatcctgattcccggacagacattacctcttcagctttttcaccctcaagaagtcagtatggtgcggaatttaattcagaaagatagaacctttgctgttcttgcatacagcaatgtacaggaaagggaagcacagtttggaacaacagcagagatatatgcctatcgagaagaacaggattttggaattgagatagtgaaagtgaaagcaattggaagacaaaggttcaaagtccttgagctaagaacacagtcagatggaatccagcaagctaaagtgcaaattcttcccgaatgtgtgttgccttcaaccatgtctgcagttcaattagaatccctcaataagtgccagatatttccttcaaaacctgtctcaagagaagaccaatgttcatataaatggtggcagaaataccagaagagaaagtttcattgtgcaaatctaacttcatggcctcgctggctgtattccttatatgatgctgagaccttaatggacagaatcaagaaacagctacgtgaatgggatgaaaatctaaaagatgattctcttccttcaaatccaatagatttttcttacagagtagctgcttgtcttcctattgatgatgtattgagaattcagctccttaaaattggcagtgctatccagcgacttcgctgtgaattagacattatgaataaatgtacttccctttgctgtaaacaatgtcaagaaacagaaataacaaccaaaaatgaaatattcagtttatccttatgtgggccgatggcagcttatgtgaatcctcatggatatgtgcatgagacacttactgtgtataaggcttgcaacttgaatctgataggccggccttctacagaacacagctggtttcctgggtatgcctggactgttgcccagtgtaagatctgtgcaagccatattggatggaagtttacggccaccaaaaaagacatgtcacctcaaaaattttggggcttaacgcgatctgctctgttgcccacgatcccagacactgaagatgaaataagtccagacaaagtaatactttgcttgtaa

SEQ ID NO: 7 - DNA, 1261 bp, Artificial Sequence
  cDNA sequence encoding a fragment from Glu24 to the stop codon of human CRBN isoform 1 or a fragment from Glu23 to the stop codon of human CRBN isoform 2
agagagtgaggaagaagatgaaatggaagttgaagaccaggatagtaaagaagccaaaaaaccaaacatcataaattttgacaccagtctgccgacatcacatacatacctaggtgctgatatggaagaatttcatggcaggactttgcacgatgacgacagctgtcaggtgattccagttcttccacaagtgatgatgatcctgattcccggacagacattacctcttcagctttttcaccctcaagaagtcagtatggtgcggaatttaattcagaaagatagaacctttgctgttcttgcatacagcaatgtacaggaaagggaagcacagtttggaacaacagcagagatatatgcctatcgagaagaacaggattttggaattgagatagtgaaagtgaaagcaattggaagacaaaggttcaaagtccttgagctaagaacacagtcagatggaatccagcaagctaaagtgcaaattcttcccgaatgtgtgttgccttcaaccatgtctgcagttcaattagaatccctcaataagtgccagatatttccttcaaaacctgtctcaagagaagaccaatgttcatataaatggtggcagaaataccagaagagaaagtttcattgtgcaaatctaacttcatggcctcgctggctgtattccttatatgatgctgagaccttaatggacagaatcaagaaacagctacgtgaatgggatgaaaatctaaaagatgattctcttccttcaaatccaatagatttttcttacagagtagctgcttgtcttcctattgatgatgtattgagaattcagctccttaaaattggcagtgctatccagcgacttcgctgtgaattagacattatgaataaatgtacttccctttgctgtaaacaatgtcaagaaacagaaataacaaccaaaaatgaaatattcagtttatccttatgtgggccgatggcagcttatgtgaatcctcatggatatgtgcatgagacacttactgtgtataaggcttgcaacttgaatctgataggccggccttctacagaacacagctggtttcctgggtatgcctggactgttgcccagtgtaagatctgtgcaagccatattggatggaagtttacggccaccaaaaaagacatgtcacctcaaaaattttggggcttaacgcgatctgctctgttgcccacgatcccagacactgaagatgaaataagtccagacaaagtaatactttgcttgtaa

SEQ ID NO: 8 - DNA, 6282 bp, Artificial Sequence
  nucleic acid sequence of targeting construct
aagaacagctcacacttgatagaataccacttctagaaagtagcgttgtgttttgtttcttcagactttcatctctgcccttggcagcatcatgttatcaggtggatcagcttagctttcatttcatttcaaaaaaaaaagtgcaggtagagttcttaagatatctccttttgccaggcagtggtggcgcactcctttaatcccagcacttgggaggcagaggcaggcagatttctgagttcgaggccagcctggtctacagagtgagttccaggacagccagggctacatagagaaaccctgtctccaaaaactcgaaaaacagaaaagaaaagaaaaaaaaaaaagacatctcctttaaaatgtattttctttgggccaactttatttttaaattgagaatgacaaagcgatgttttatgaaaaataattgcaaacatttcacgtttaaatatgacggtgagccaggttttaatggtattttttttcccagtttcattaacagacctttcttgcctgcttgtgttttccttgctttctttttcacagagaaactttgtagctaaagtctgaaagaacctcatagattactttgttcaagccttcattgttttttttttcaaatgaaaaaacagctttaatcaattggaattcattgtgtaaggtgtcaggattagtagtgatggagaagataagactcatccatgcaggagatgggcctaattcagccacgtcagtcgttaggctggacctagtgatctgctttccaaccgtgtacggtgtaactgcggggcaggggcgagggggtttacagagaaggaagctggcggctgtttctgaccagaaatcaaggggaacatcagcccctgggtcaggctgactgtacgtacccttgatgtgcggtgaggaataggcgttgtccctagcagaactctaatagagaatgacatctattccctattgagggatgctgtgtaaagtcctgataaggaagacagaacatccagcatgcgtgtaccacaggcagcaaaggagccatacctaaatatagcatggtgtcctggaggggtaacaggaaatggagaatagctgaaaatcaaaggcaatccaaataagataaggcatttagttaacagtaatgtgccaatatcgacgacttagttgtcacaagaataccagatgcatggaccatgctaacaatggaggaagatagtcttggcatgctagaattctatttttccaacattccaggaaatcttaaagtgtcctaagatagttgattgttaaaaacagggaaaaaagaaaggaaaggaaaagaaaggaaaaggcgccatgacagaaagagcacagacccagcctctgccgctgtctctgcacagctttccttttaagagtgtctttcttcaattcagggtgtgtgaatggaaccagaactgacttgcttttttcttttctttttttttttttttaatgaatctcattttttccctctattattctccttcagcagagagtgaggaagaagatgaaatggaagttgaagaccaggatagtaaagaagccaaaaaaccaaacatcataaattttgacaccagtctgccgacatcacatacatacctaggtgctgatatggaagaatttcatggcaggactttgcacgatgacgacagctgtcaggtgattccagttcttccacaagtgatgatgatcctgattcccggacagacattacctcttcagctttttcaccctcaagaagtcagtatggtgcggaatttaattcagaaagatagaacctttgctgttcttgcatacagcaatgtacaggaaagggaagcacagtttggaacaacagcagagatatatgcctatcgagaagaacaggattttggaattgagatagtgaaagtgaaagcaattggaagacaaaggttcaaagtccttgagctaagaacacagtcagatggaatccagcaagctaaagtgcaaattcttcccgaatgtgtgttgccttcaaccatgtctgcagttcaattagaatccctcaataagtgccagatatttccttcaaaacctgtctcaagagaagaccaatgttcatataaatggtggcagaaataccagaagagaaagtttcattgtgcaaatctaacttcatggcctcgctggctgtattccttatatgatgctgagaccttaatggacagaatcaagaaacagctacgtgaatgggatgaaaatctaaaagatgattctcttccttcaaatccaatagatttttcttacagagtagctgcttgtcttcctattgatgatgtattgagaattcagctccttaaaattggcagtgctatccagcgacttcgctgtgaattagacattatgaataaatgtacttccctttgctgtaaacaatgtcaagaaacagaaataacaaccaaaaatgaaatattcagtttatccttatgtgggccgatggcagcttatgtgaatcctcatggatatgtgcatgagacacttactgtgtataaggcttgcaacttgaatctgataggccggccttctacagaacacagctggtttcctgggtatgcctggactgttgcccagtgtaagatctgtgcaagccatattggatggaagtttacggccaccaaaaaagacatgtcacctcaaaaattttggggcttaacgcgatctgctctgttgcccacgatcccagacactgaagatgaaataagtccagacaaagtaatactttgcttgtaagtgcacctagagctcgctgatcagcctcgactgtgccttctagttgccagccatctgttgtttgcccctcccccgtgccttccttgaccctggaaggtgccactcccactgtcctttcctaataaaatgaggaaattgcatcgcattgtctgagtaggtgtcattctattctggggggtggggtggggcaggacagcaagggggaggattgggaagacaatagcaggcatgctggggatgcggtgggctctatggcttctgaggcggaaagaaccagctggggctcgactagagcttgcggaacccttcgtatgtggtttagtcattgagcaaatgcagtatgcggacctttatctatggctggaatttggtaccttttgctagcataacttcgtatagcatacattatacgaagttatcctaggtaattctaccgggtaggggaggcgcttttcccaaggcagtctggagcatgcgctttagcagccccgctgggcacttggcgctacacaagtggcctctggcctcgcacacattccacatccaccggtaggcgccaaccggctccgttctttggtggccccttcgcgccaccttctactcctcccctagtcaggaagttcccccccgccccgcagctcgcgtcgtgcaggacgtgacaaatggaagtagcacgtctcactagtctcgtgcagatggacagcaccgctgagcaatggaagcgggtaggcctttggggcagcggccaatagcagctttgctccttcgctttctgggctcagaggctgggaaggggtgggtccgggggcgggctcaggggcgggctcaggggcggggcgggcgcccgaaggtcctccggaggcccggcattctgcacgcttcaaaagcgcacgtctgccgcgctgttctcctcttcctcatctccgggcctttcgacctgcagcctgttgacaattaatcatcggcatagtatatcggcatagtataatacgacaaggtgaggaactaaaccagatctgccaccatgattgaacaagatggattgcacgcaggttctccggccgcttgggtggagaggctattcggctatgactgggcacaacagacaatcggctgctctgatgccgccgtgttccggctgtcagcgcaggggcgcccggttctttttgtcaagaccgacctgtccggtgccctgaatgaactgcaggacgaggcagcgcggctatcgtggctggccacgacgggcgttccttgcgcagctgtgctcgacgttgtcactgaagcgggaagggactggctgctattgggcgaagtgccggggcaggatctcctgtcatctcaccttgctcctgccgagaaagtatccatcatggctgatgcaatgcggcggctgcatacgcttgatccggctacctgcccattcgaccaccaagcgaaacatcgcatcgagcgagcacgtactcggatggaagccggtcttgtcgatcaggatgatctggacgaagagcatcaggggctcgcgccagccgaactgttcgccaggctcaaggcgcgcatgcccgacggcgaggatctcgtcgtgacccatggcgatgcctgcttgccgaatatcatggtggaaaatggccgcttttctggattcatcgactgtggccggctgggtgtggcggaccgctatcaggacatagcgttggctacccgtgatattgctgaagagcttggcggcgaatgggctgaccgcttcctcgtgctttacggtatcgccgctcccgattcgcagcgcatcgccttctatcgccttcttgacgagttcttctgacttaagaacttgtttattgcagcttataatggttacaaataaagcaatagcatcacaaatttcacaaataaagcatttttttcactgcattctagttgtggtttgtccaaactcatcaatgtatcttatcatgtctgcaattgataacttcgtatagcatacattatacgaagttatgaattcttttctcgagcctaagtgcagggagccacactaggggactagtgcaggggactgactagagggttcctgcatattcgctgaccctagaatccgtgcatgagaacagacttattttccagtgcatagcatgtaattttagaaatggaagccgtgtcgtactatatcctcatgtgattcttgactattttctaatatgtaagctgatatgtaaacattaaagctaacatatagctttatgtttaaacttatcttgggagggactctttgaggaattgtcttcctctgaagggttctgctagtaactgagccattaagtgttcttaatgttgtttcagaactgctgggatgtggggcggtattataggtactaaaattctgtcctatgctttgtcagttttggacatagaggagttttggtgaaaatattttgaattacaaaataatgatcgattcttgataaaaattgggagttctaataggaaatactagatcaaaaattagagtttgatggaggcatgcttatataacagattatttaaataaacatgtgctctgtttagtgttttcctctgctttattctttagtaggttgacgtgtagtaagtgtgtgtcttgactctgtgctcttgagtagtacctgggagctgatatggaggagttccacgggagaactttgcatgacgacgacagctgccaggtgatcccagtccttcctgaggtgctgatgatcctgattcctgggcagacactcccactgcagctctctcacccacaggaagtcagcatggtgcggaacttaatccagaaagacaggacctttgcagtccttgcatacaggtaagagattagacagatctgcttaccaccctgccaaagtcagtgcgacagctaaagccaacggggatttgcagatactggacaggagtgtgaagcaaacggtcttgtgtcacattttcagtgtttcgctgtttttacagtgtagctgtgtttggctcttgaaaaacttccactcacttaatggaaaacctccctgttcagaactgtctttatttaaaaatagctaagttttaaaattttcaataaaggttacttttctaaagtgaagctgttcttcagtagcctgtggcaaatgagggaaccgtggtggaggcaggaaatggaaacaggaaacctcccatcacccccgctgaccctcccctcagacagtcacagtgctgccagttagtgcgaccatcattgcctgccaaagtgaaaggatgctcattttgtgaaataacgatttaaaacttcttagcactggttatctcagtgaagcctaaaagtctacctttattctaaaatatgctgtttgccttccggggccttgtgtgtcagcttcctagtgagggttagctgctgtaattgtcacagtgtttgcccgatctgtgtcgcttttgccacctttacataattatgagccagagctgaaaactctgtccatttttgtctttgaagtaatgtgcaagaaaggg

SEQ ID NO: 9 - DNA, 50 bp, Artificial Sequence
  TALEN 1 targeting sequence
tatgcggacctttatctatggctggaatttcctaagtgcagggagccaca

SEQ ID NO: 10 - DNA, 49 bp, Artificial Sequence
  TALEN 2 targeting sequence
tgcagtatgcggacctttatctatggctggaatttcctaagtgcaggga

SEQ ID NO: 11 - DNA, 48 bp, Artificial Sequence
  TALEN 3 targeting sequence
tctgccaacctcacatacagtatgtggtttagtcattgagcaaatgca

SEQ ID NO: 12 - DNA, 20 bp, Artificial Sequence
  forward primer for detecting CRBN 5-prime targeting
ctgcattaccggggttttta

SEQ ID NO: 13 - DNA, 20 bp, Artificial Sequence
  reverse primer for detecting CRBN 5-prime targeting
gctgttgttccaaactgtgc

SEQ ID NO: 14 - DNA, 20 bp, Artificial Sequence
  forward primer for detecting CRBN 3-prime targeting
cggaccgctatcaggacata

SEQ ID NO: 15 - DNA, 20 bp, Artificial Sequence
  reverse primer for detecting CRBN 3-prime targeting
gccttccaattgctttcact

SEQ ID NO: 16 - DNA, 20 bp, Artificial Sequence
  forward primer for genotyping
tgtgttgccttcaaccatgt

SEQ ID NO: 17 - DNA, 20 bp, Artificial Sequence
  reverse primer for genotyping
cagcatgcctgctattgtct